European Patent Specification EP 3 805 375 B1, published June 18, 2025. Title: METHOD FOR IN VITRO REPROGRAMMING OF FIBROBLASTS INTO SERTOLI CELLS AND APPLICATION THEREOF. Applicant: TSINGHUA UNIVERSITY. The sequence listing filed with the application follows.

SEQUENCE LISTING (3 sequences)

SEQ ID NO: 1 - DNA, 1558 bp, Artificial sequence
tgctgaacctttctccgtctctctagttcttcctccagttccactttaagatggagaagcccccggctccacccagcctccctgctggcccccctggggtgaagcggcctccacccccgctgatgaacggtctgccccctcggccaccgctgcctgagtctttgccaccgcccccgccaggaggcctgcctctgccacccatgccccccacagggcctgcgccctcagggcccccgggaccaccccagctacccccgccagctccaggggtccaccccccggccccagtggtgcatccccctgcatctggggtccatcccccagctcctggcgtccaccccccagctcctggcgtccatcccccagcccctggggtccacccaccaacctctggggtccaccccccagctcctggagtccaccctccagcccccggggttcacccaccagcccccggagtccacccaccagcccctggggttcacccaccagccccaggggtccatcctcccccatcagcgggggttcacccccaggccccgggggtgcacccagcagcccccgccgttcaccctcaggccccaggggtgcacccaccagccccagggatgcaccctcaggccccgggggtccacccccaacctcccggggtccatccgtcggctcctggggtccaccctcagcctccgggagttcacccctcaaatcctggggtgcaccccccaactcccatgcccccaatgctgaggcccccacttccctccgaaggcccagggaacatacctccccctcccccaaccaactgagaagctgctccctcccccagcaagcccagcgccaggtgctcttgccttttcccactgagagaaggctgctcttttgtactgccccccgctcattaaacagcctcccccagccctgagtgcactgatgtccgcagcgccgccctactgtgtcagtgtgtgtgggagtgccaggcacagcaccatcccccagtttgggccgactggggagggcctggggcccgccaggagacacctgtgggaggcctgagagatggctgtaccttggagatggcctggtggaggacagaccccaccagccagctaggaggggatctggggtcctgttctggggagggaagagcagactccacgatatccttggggtctccagatagcccaccaggggtggggagggtgagcagggacagggcgcccccactgacttgggaccctcctcctccaggcccacacctcagcacccaggacatctgggccccccgcccccagcgctgtctagtttggttgcctggccgtcactcccagcctggttcccactcctgtgtcttctggggatggccctcaaggacggcatgttgacacatcaggcccagctctatcactggggagggagataggctgccagggacagaaagggctctttgagaaggccactctgcctggagtgggggcgccgggcactgtcccccaaggtcgcggcagaggagataggggtctgtcctgcacaaacaccccaccttccactcggctcactt

SEQ ID NO: 2 - DNA, 1172 bp, Artificial sequence
gtgcccgtcagtgggcagagcgcacatcgcccacagtccccgagaagttggggggaggggtcggcaattgaaccggtgcctagagaaggtggcgcggggtaaactgggaaagtgatgtcgtgtactggctccgcctttttcccgagggtgggggagaaccgtatataagtgcagtagtcgccgtgaacgttctttttcgcaacgggtttgccgccagaacacaggtaagtgccgtgtgtggttcccgcgggcctggcctctttacgggttatggcccttgcgtgccttgaattacttccacctggctgcagtacgtgattcttgatcccgagcttcgggttggaagtgggtgggagagttcgaggccttgcgcttaaggagccccttcgcctcgtgcttgagttgaggcctggcctgggcgctggggccgccgcgtgcgaatctggtggcaccttcgcgcctgtctcgctgctttcgataagtctctagccatttaaaatttttgatgacctgctgcgacgctttttttctggcaagatagtcttgtaaatgcgggccaagatctgcacactggtatttcggtttttggggccgcgggcggcgacggggcccgtgcgtcccagcgcacatgttcggcgaggcggggcctgcgagcgcggccaccgagaatcggacgggggtagtctcaagctggccggcctgctctggtgcctggcctcgcgccgccgtgtatcgccccgccctgggcggcaaggctggcccggtcggcaccagttgcgtgagcggaaagatggccgcttcccggccctgctgcagggagctcaaaatggaggacgcggcgctcgggagagcgggcgggtgagtcacccacacaaaggaaaagggcctttccgtcctcagccgtcgcttcatgtgactccacggagtaccgggcgccgtccaggcacctcgattagttctcgagcttttggagtacgtcgtctttaggttggggggaggggttttatgcgatggagtttccccacactgagtgggtggagactgaagttaggccagcttggcacttgatgtaattctccttggaatttgccctttttgagtttggatcttggttcattctcaagcctcagacagtggttcaaagtttttttcttccatttcaggtgtcgtga

SEQ ID NO: 3 - DNA, 726 bp, Artificial sequence
caggtgctcttgccttttcccactgagagaaggctgctcttttgtactgccccccgctcattaaacagcctcccccagccctgagtgcactgatgtccgcagcgccgccctactgtgtcagtgtgtgtgggagtgccaggcacagcaccatcccccagtttgggccgactggggagggcctggggcccgccaggagacacctgtgggaggcctgagagatggctgtaccttggagatggcctggtggaggacagaccccaccagccagctaggaggggatctggggtcctgttctggggagggaagagcagactccacgatatccttggggtctccagatagcccaccaggggtggggagggtgagcagggacagggcgcccccactgacttgggaccctcctcctccaggcccacacctcagcacccaggacatctgggccccccgcccccagcgctgtctagtttggttgcctggccgtcactcccagcctggttcccactcctgtgtcttctggggatggccctcaaggacggcatgttgacacatcaggcccagctctatcactggggagggagataggctgccagggacagaaagggctctttgagaaggccactctgcctggagtgggggcgccgggcactgtcccccaaggtcgcggcagaggagataggggtctgtcctgcacaaacaccccaccttccactcggctcacttaaggca